European Patent Specification EP 3 383 405 B1, published June 12, 2024. Title: Antibiotic FIIRV104/18 complex and the isolated individual factors thereof. Applicant: Fondazione Istituto Insubrico di Ricerca per la Vita (FIIRV). The sequence listing filed with the application follows.

SEQUENCE LISTING (1 sequence)

SEQ ID NO: 1 - DNA, 1294 bp, Dactylosporangium sp.
  gene (1)..(1294)
ggctttgggataaccctcggaaacgggggctaataccggatattcatgctggacggcatcgtttggtgtggaaagtttttcggcttgggatgggctcgcggcctatcagcttgttggtggggtgatggcctaccaaggcgacgacgggtagccggcctgagagggcgaccggccacactgggactgagacacggcccagactcctacgggaggcagcagtggggaatattgcacaatgggcggaagcctgatgcagcgacgccgcgtgagggatgaaggccttcgggttgtaaacctctttcgacagggacgaagcgtgagtgacggtacctggagaagaagcgccggccaactacgtgccagcagccgcggtaagacgtagggcgcgagcgttgtccggatttattgggcgtaaagagctcgtaggcggcttgttgcgtcagctgtgaaaacccgcagctcaactgtgggcttgcagctgatacgggcaggcttgagttcggtaggggagactggaattcctggtgtagcggtgaaatgcgcagatatcaggaggaacaccggtggcgaaggcgggtctctgggccgatactgacgctgaggagcgaaagcgtggggagcgaacaggattagataccctggtagtccacgctgtaaacgttgggcgctaggtgtggggggcctctccggttctctgtgccgcagctaacgcattaagcgccccgcctggggagtacggccgcaaggctaaaactcaaaggaattgacgggggcccgcacaagcggcggagcatgcggattaattcgatgcaacgcgaagaaccttacctgggtttgacatgttcggtaatccggcagagatgtcgggtccttcggggccgttcacaggtggtgcatggctgtcgtcagctcgtgtcgtgagatgttgggttaagtcccgcaacgagcgcaacccttgttcgatgttgccagcggttcggccggggactcatcgaagactgccggggtcaactcggaggaaggtggggatgacgtcaagtcatcatgccccttatgtccagggcttcacgcatgctacaatggccggtacaaagggctgcgataccgtgaggtggagcgaatcccaaaaagccggtctcagttcggatcggggtctgcaactcgaccccgtgaagtcggagtcgctagtaatcgcagatcagcaatgctgcggtgaatacgttcccgggccttgtacacaccgcccgtcacgtcacgaaagtcggcaacacccgaagccggtggcccaaccctt